European Patent Specification EP 3 453 759 B1, published August 30, 2023. Title: Platelet Production Stimulators and Method for Producing Platelets with the Same. Applicant: Kyoto University Megakaryon Corporation. The sequence listing filed with the application follows.

SEQUENCE LISTING (7 sequences)

SEQ ID NO: 1 - DNA, 115 bp, Artificial Sequence
  Target vector
ggatccgtgtgagagaagctgtgccggttttagagctagaaatagcaagttaaaataaggctagtccgttatcaacttgaaaaagtggcaccgagtcggtgctttttttgaattc

SEQ ID NO: 2 - DNA, 20 bp, Artificial Sequence
  TUBB1 insert check Fw
gatgctttactggtgccctt

SEQ ID NO: 3 - DNA, 20 bp, Artificial Sequence
  TUBB1 insert check Rv
aagagatggcagtgctgcat

SEQ ID NO: 4 - DNA, 20 bp, Artificial Sequence
  5-1 insert check Fw
tgctttactggtgcccttct

SEQ ID NO: 5 - DNA, 20 bp, Artificial Sequence
  5-1.2 insert check Rv
aagtcgtgctgcttcatgtg

SEQ ID NO: 6 - DNA, 20 bp, Artificial Sequence
  3-1.2 insert check Fw
gcaacctccccttctacgag

SEQ ID NO: 7 - DNA, 20 bp, Artificial Sequence
  3-2 insert check Rv
tcggagcattttcccattac